European Patent Specification EP 3 474 885 B1, published May 10, 2023. Title: MICROBIOME PROTECTION FROM ORAL ANTIBIOTICS. Applicant: Synthetic Biologics, Inc. KALEKO, Michael CONNELLY, Sheila. The sequence listing filed with the application follows.

SEQUENCE LISTING (7 sequences)

SEQ ID NO: 1 - protein, 263 aa, Bacillus licheniformis
EMKDDFAKLEEQFDAKLGIFALDTGTNRTVAYRPDERFAFASTIKALTVGVLLQQKSIEDLNQRITYTRDDLVNYNPITEKHVDTGMTLKELADASLRYSDNAAQNLILKQIGGPESLKKELRKIGDEVTNPERFEPELNEVNPGETQDTSTARALVTSLRAFALEDKLPSEKRELLIDWMKRNTTGDALIRAGVPDGWEVADKTGAASYGTRNDIAIIWPPKGDPVVLAVLSSRDKKDAKYDDKLIAEATKVVMKALNMNGK

SEQ ID NO: 2 - DNA, 792 bp, Bacillus licheniformis
gagatgaaagatgattttgcaaaacttgaggaacaatttgatgcaaaactcgggatctttgcattggatacaggtacaaaccggacggtagcgtatcggccggatgagcgttttgcttttgcttcgacgattaaggctttaactgtaggcgtgcttttgcaacagaaatcaatagaagatctgaaccagagaataacatatacacgtgatgatcttgtaaactacaacccgattacggaaaagcacgttgatacgggaatgacgctcaaagagcttgcggatgcttcgcttcgatatagtgacaatgcggcacagaatctcattcttaaacaaattggcggacctgaaagtttgaaaaaggaactgaggaagattggtgatgaggttacaaatcccgaacgattcgaaccagagttaaatgaagtgaatccgggtgaaactcaggataccagtacagcaagagcacttgtcacaagccttcgagcctttgctcttgaagataaacttccaagtgaaaaacgcgagcttttaatcgattggatgaaacgaaataccactggagacgccttaatccgtgccggtgtgccggacggttgggaagtggctgataaaactggagcggcatcatatggaacccggaatgacattgccatcatttggccgccaaaaggagatcctgtcgttcttgcagtattatccagcagggataaaaaggacgccaagtatgatgataaacttattgcagaggcaacaaaggtggtaatgaaagccttaaacatgaacggcaaataa

SEQ ID NO: 3 - protein, 299 aa, Bacillus licheniformis
MIQKRKRTVSFRLVLMCTLLFVSLPITKTSAQASKTEMKDDFAKLEEQFDAKLGIFALDTGTNRTVAYRPDERFAFASTIKALTVGVLLQQKSIEDLNQRITYTRDDLVNYNPITEKHVDTGMTLKELADASLRYSDNAAQNLILKQIGGPESLKKELRKIGDEVTNPERFEPELNEVNPGETQDTSTARALVTSLRAFALEDKLPSEKRELLIDWMKRNTTGDALIRAGVPDGWEVADKTGAASYGTRNDIAIIWPPKGDPVVLAVLSSRDKKDAKYDDKLIAEATKVVMKALNMNGK

SEQ ID NO: 4 - DNA, 900 bp, Bacillus licheniformis
atgattcaaaaacgaaagcggacagtttcgttcagacttgtgcttatgtgcacgctgttatttgtcagtttgccgattacaaaaacatcagcgcaagcttccaagacggagatgaaagatgattttgcaaaacttgaggaacaatttgatgcaaaactcgggatctttgcattggatacaggtacaaaccggacggtagcgtatcggccggatgagcgttttgcttttgcttcgacgattaaggctttaactgtaggcgtgcttttgcaacagaaatcaatagaagatctgaaccagagaataacatatacacgtgatgatcttgtaaactacaacccgattacggaaaagcacgttgatacgggaatgacgctcaaagagcttgcggatgcttcgcttcgatatagtgacaatgcggcacagaatctcattcttaaacaaattggcggacctgaaagtttgaaaaaggaactgaggaagattggtgatgaggttacaaatcccgaacgattcgaaccagagttaaatgaagtgaatccgggtgaaactcaggataccagtacagcaagagcacttgtcacaagccttcgagcctttgctcttgaagataaacttccaagtgaaaaacgcgagcttttaatcgattggatgaaacgaaataccactggagacgccttaatccgtgccggtgtgccggacggttgggaagtggctgataaaactggagcggcatcatatggaacccggaatgacattgccatcatttggccgccaaaaggagatcctgtcgttcttgcagtattatccagcagggataaaaaggacgccaagtatgatgataaacttattgcagaggcaacaaaggtggtaatgaaagccttaaacatgaacggcaaataa

SEQ ID NO: 5 - protein, 262 aa, Artificial Sequence
  Synthetic sequence
EMKDDFAKLEEQFDAKLGIFALDTGTNRTVAYRPDERFAFASTIKALTVGVLLQQKSIEDLNQRITTRDDLVNYNPITEKHVDTGMTLKELADASLRYSDNAAQNLILKQIGGPESLKKELRKIGDEVTNPERFEPELNEVNPGETQDTSTARALVTSLRAFALEDKLPSEKRELLIDWMKRNTTGDALIRAGVPDGWEVGDKTGSGDYGTRNDIAIIWPPKGDPVVLAVLSSRDKKDAKYDNKLIAEATKVVMKALNMNGK

SEQ ID NO: 6 - protein, 299 aa, Artificial Sequence
  Synthetic sequence
MIQKRKRTVSFRLVLMCTLLFVSLPITKTSAQASKTEMKDDFAKLEEQFDAKLGIFALDTGTNRTVAYRPDERFAFASTIKALTVGVLLQQKSIEDLNQRITYTRDDLVNYNPITEKHVDTGMTLKELADASLRYSDNAAQNLILKQIGGPESLKKELRKIGDEVTNPERFEPELNEVNPGETQDTSTARALVTSLRAFALEDKLPSEKRELLIDWMKRNTTGDALIRAGVPDGWEVGDKTGSGDYGTRNDIAIIWPPKGDPVVLAVLSSRDKKDAKYDNKLIAEATKVVMKALNMNGK

SEQ ID NO: 7 - DNA, 900 bp, Artificial Sequence
  Synthetic sequence
atgattcaaaaacgaaagcggacagtttcgttcagacttgtgcttatgtgcacgctgttatttgtcagtttgccgattacaaaaacatcagcgcaagcttccaagacggagatgaaagatgattttgcaaaacttgaggaacaatttgatgcaaaactcgggatctttgcattggatacaggtacaaaccggacggtagcgtatcggccggatgagcgttttgcttttgcttcgacgattaaggctttaactgtaggcgtgcttttgcaacagaaatcaatagaagatctgaaccagagaataacatatacacgtgatgatcttgtaaactacaacccgattacggaaaagcacgttgatacgggaatgacgctcaaagagcttgcggatgcttcgcttcgatatagtgacaatgcggcacagaatctcattcttaaacaaattggcggacctgaaagtttgaaaaaggaactgaggaagattggtgatgaggttacaaatcccgaacgattcgaaccagagttaaatgaagtgaatccgggtgaaactcaggataccagtacagcaagagcacttgtcacaagccttcgagcctttgctcttgaagataaacttccaagtgaaaaacgcgagcttttaatcgattggatgaaacgaaataccactggagacgccttaatccgtgccggtgtgccggacggttgggaagtgggtgataaaactggaagcggagattatggaacccggaatgacattgccatcatttggccgccaaaaggagatcctgtcgttcttgcagtattatccagcagggataaaaaggacgccaagtatgataataaacttattgcagaggcaacaaaggtggtaatgaaagccttaaacatgaacggcaaataa